European Patent Application EP 4 782 540 A1, published July 29, 2026. Title: 1本鎖ポリヌクレオチド. Applicant: 国立大学法人東海国立大学機構. The sequence listing filed with the application follows.

SEQUENCE LISTING (43 sequences)

SEQ ID NO: 1 - DNA, 14 bp, synthetic construct
  source 1..14: mol_type = other DNA
catggtgtggcaac

SEQ ID NO: 2 - DNA, 18 bp, synthetic construct
  source 1..18: mol_type = other DNA
aggtaagctccattgtgc

SEQ ID NO: 3 - DNA, 22 bp, synthetic construct
  source 1..22: mol_type = other DNA
ggtgcatggtgtggcaacaggt

SEQ ID NO: 4 - DNA, 21 bp, synthetic construct
  source 1..21: mol_type = other DNA
ggtgcatggtgtggcaacagg

SEQ ID NO: 5 - DNA, 100 bp, synthetic construct
  source 1..100: mol_type = other DNA
gtttttgtaggctccaaaaccaaggagggagtggtgcatggtgtggcaacaggtaagctccattgtgcttatatccaaagatgatatttaaagtatctag

SEQ ID NO: 6 - DNA, 18 bp, synthetic construct
  source 1..18: mol_type = other DNA
agcctacaaaaacaaatt

SEQ ID NO: 7 - DNA, 18 bp, synthetic construct
  source 1..18: mol_type = other DNA
tttggagcctacaaaaac

SEQ ID NO: 8 - DNA, 18 bp, synthetic construct
  source 1..18: mol_type = other DNA
ttggttttggagcctaca

SEQ ID NO: 9 - DNA, 18 bp, synthetic construct
  source 1..18: mol_type = other DNA
cctccttggttttggagc

SEQ ID NO: 10 - DNA, 18 bp, synthetic construct
  source 1..18: mol_type = other DNA
cactccctccttggtttt

SEQ ID NO: 11 - DNA, 18 bp, synthetic construct
  source 1..18: mol_type = other DNA
tgcaccactccctccttg

SEQ ID NO: 12 - DNA, 18 bp, synthetic construct
  source 1..18: mol_type = other DNA
caccatgcaccactccct

SEQ ID NO: 13 - DNA, 18 bp, synthetic construct
  source 1..18: mol_type = other DNA
tgccacaccatgcaccac

SEQ ID NO: 14 - DNA, 18 bp, synthetic construct
  source 1..18: mol_type = other DNA
cctgttgccacaccatgc

SEQ ID NO: 15 - DNA, 18 bp, synthetic construct
  source 1..18: mol_type = other DNA
gcttacctgttgccacac

SEQ ID NO: 16 - DNA, 18 bp, synthetic construct
  source 1..18: mol_type = other DNA
atggagcttacctgttgc

SEQ ID NO: 17 - DNA, 18 bp, synthetic construct
  source 1..18: mol_type = other DNA
gcacaatggagcttacct

SEQ ID NO: 18 - DNA, 23 bp, synthetic construct
  source 1..23: mol_type = other DNA
atggatgtattcatgaaaggact

SEQ ID NO: 19 - DNA, 20 bp, synthetic construct
  source 1..20: mol_type = other DNA
ttaggcttcaggttcgtagt

SEQ ID NO: 20 - DNA, 20 bp, synthetic construct
  source 1..20: mol_type = other DNA
gagtcaacggatttggtcgt

SEQ ID NO: 21 - DNA, 20 bp, synthetic construct
  source 1..20: mol_type = other DNA
ttgattttggagggatctcg

SEQ ID NO: 22 - DNA, 20 bp, synthetic construct
  source 1..20: mol_type = other DNA
ccttcttcattcttgcccaa

SEQ ID NO: 23 - DNA, 21 bp, synthetic construct
  source 1..21: mol_type = other DNA
agagggtgttctctatgtagg

SEQ ID NO: 24 - DNA, 21 bp, synthetic construct
  source 1..21: mol_type = other DNA
agagggtgttctctatgtagt

SEQ ID NO: 25 - DNA, 19 bp, synthetic construct
  source 1..19: mol_type = other DNA
cttcttcattcttgcccaa

SEQ ID NO: 26 - DNA, 20 bp, synthetic construct
  source 1..20: mol_type = other DNA
cgtcccgtagacaaaatggt

SEQ ID NO: 27 - DNA, 20 bp, synthetic construct
  source 1..20: mol_type = other DNA
gaatttgccgtgagtggagt

SEQ ID NO: 28 - DNA, 18 bp, synthetic construct
  source 1..18: mol_type = other DNA
cactaccagctgttccgc

SEQ ID NO: 29 - DNA, 18 bp, synthetic construct
  source 1..18: mol_type = other DNA
accccggcctcactgtta

SEQ ID NO: 30 - DNA, 18 bp, synthetic construct
  source 1..18: mol_type = other DNA
ttgccacaccatgcacca

SEQ ID NO: 31 - DNA, 18 bp, synthetic construct
  source 1..18: mol_type = other DNA
gttgccacaccatgcacc

SEQ ID NO: 32 - DNA, 18 bp, synthetic construct
  source 1..18: mol_type = other DNA
tgttgccacaccatgcac

SEQ ID NO: 33 - DNA, 18 bp, synthetic construct
  source 1..18: mol_type = other DNA
ctgttgccacaccatgca

SEQ ID NO: 34 - DNA, 18 bp, synthetic construct
  source 1..18: mol_type = other DNA
acctgttgccacaccatg

SEQ ID NO: 35 - DNA, 18 bp, synthetic construct
  source 1..18: mol_type = other DNA
tacctgttgccacaccat

SEQ ID NO: 36 - DNA, 18 bp, synthetic construct
  source 1..18: mol_type = other DNA
ttacctgttgccacacca

SEQ ID NO: 37 - DNA, 18 bp, synthetic construct
  source 1..18: mol_type = other DNA
cttacctgttgccacacc

SEQ ID NO: 38 - RNA, 15 nt, synthetic construct
  source 1..15: mol_type = other RNA
gcatggtgtggcaac

SEQ ID NO: 39 - DNA, 21 bp, synthetic construct
  source 1..21: mol_type = other DNA
agagggtgttctctatgtagg

SEQ ID NO: 40 - DNA, 21 bp, synthetic construct
  source 1..21: mol_type = other DNA
agagggtgttctctatgtagt

SEQ ID NO: 41 - DNA, 19 bp, synthetic construct
  source 1..19: mol_type = other DNA
cttcttcattcttgcccaa

SEQ ID NO: 42 - DNA, 20 bp, synthetic construct
  source 1..20: mol_type = other DNA
cgtcccgtagacaaaatggt

SEQ ID NO: 43 - DNA, 20 bp, synthetic construct
  source 1..20: mol_type = other DNA
gaatttgccgtgagtggagt